European Patent Application EP 4 733 406 A1, published April 29, 2026. Title: Verfahren zur Herstellung von 2,5-Furandicarbonsäure. Applicant: Annikki GmbH. Application EP. The sequence listing filed with the application follows.

SEQUENCE LISTING (16 sequences)

SEQ ID NO: 1 - DNA, 1410 bp, Pseudomonas nitroreducens
  source 1..1410: mol_type = genomic DNA
atgtcacgctatgaactgctgatcgatggtcgcctgcaggcggccgagcactacgaccgggtgatcgacccggccagcgaagaaatcgttggcgaagccgcccgcgccagcctggagcaggtcgacgcggcggtggatgccgcacaccgcgccttcccggcctgggccaccgatctcgacgtccgccgccagagcctggcccgagccgccgaacgagtacgcgagaatgcccaggcgctggccgagctgatcacccgcgaacagggtcgcccactgcgctcgaccctggaggaagtggctggcgtcgccgccactttcgagcaccacgcgcagctggagctacccgccgacacccagttgcgcgacgacggcgagcgcctggtgcgcatcacccgcaaaccgctgggggtggtcgccgcgatcaccccgtggaacgtcccgctgatcctgctggtattgaagatcgcgcctgccctgcacgccggcaacaccgtggtggccaagccctcggagcacacgccgctgtctaccctgctgctggcgcgactgctgggcgatgtgttccccgctggcgtgttcaacgtggttgccggtgcgggcgaggttggcgaacacctggtacgtcatccgcgggtgcgccacgtgaccttcaccggcagcgtcgccaccggcaagcgcctgtatgccggcgcgggggacgacctcaagcgtcttaccctggaactgggcggcaacgacgccgcgctggtactggaagacgccgacctcgacgccatcgtcgaaccgctgttctggggcgccttctggaacagcggccaggtgtgctttgcgatcaagcgcctgtacgtgcatgacagcctgttcgaaccgttactggcgaaactcgccgagcgcgcccagcgcacccgcctcggtcatgggctcgacccgcagacggaactggggccgctgaccaacgcacagcaactggaacgggtcatcgccctggtggaagacgccaaggctcacggagcacgcatccgcagcggcggcgtacggcccgacggtcccggctacttctacccgccgaccctggtcagcggcgtggcggccggcgtcgcgctggtggacgaggaacagttcggcccggtgttgccggtgatctccttccgcaacgaagaggacgccattacccaggccaacgccagccactacggcctcggcgcctcggtgtggacccgcgacctggcgcgcggcgaagccatcgccaggcggctggaggcgggcctggcctgggtcaaccagcacggccacatccagcccggcgcgcccaagggcgggcacaagtggagcgggctcggctacgaaggcgggcagcgcggctatgaggccttcagcgagctgcaggtgctgaacatttcgcggcgctaa

SEQ ID NO: 2 - protein, 469 aa, Pseudomonas nitroreducens
MSRYELLIDGRLQAAEHYDRVIDPASEEIVGEAARASLEQVDAAVDAAHRAFPAWATDLDVRRQSLARAAERVRENAQALAELITREQGRPLRSTLEEVAGVAATFEHHAQLELPADTQLRDDGERLVRITRKPLGVVAAITPWNVPLILLVLKIAPALHAGNTVVAKPSEHTPLSTLLLARLLGDVFPAGVFNVVAGAGEVGEHLVRHPRVRHVTFTGSVATGKRLYAGAGDDLKRLTLELGGNDAALVLEDADLDAIVEPLFWGAFWNSGQVCFAIKRLYVHDSLFEPLLAKLAERAQRTRLGHGLDPQTELGPLTNAQQLERVIALVEDAKAHGARIRSGGVRPDGPGYFYPPTLVSGVAAGVALVDEEQFGPVLPVISFRNEEDAITQANASHYGLGASVWTRDLARGEAIARRLEAGLAWVNQHGHIQPGAPKGGHKWSGLGYEGGQRGYEAFSELQVLNISRR

SEQ ID NO: 3 - DNA, 1410 bp, Methylovorus glucosotrophus
  source 1..1410: mol_type = genomic DNA
atgtcgacatttcatttacttattgatggccatctgcaagccagtgaccaatccgatgtggtgatcaaccccgcgaccgagctggaagtcgggcgtgccccacgtgccagcgccacccaggtcgaccaggcagtggaagccgcacatcaggcatttcatcgctgggcatcacagcctgaggtgcgccagcaggcactgctgggcgcggccgccgccattcgccagcatgccgatgccctggcacgcctgatcacgcaagagcaggggcggccattgcactttacccagggcgaggtggccggggctgctgctacctttgaacactatgccgggtttgccgcgccatcggatgtggtgctgcagcaggacgaacaaaagcgggtcagcattgagcgcaggccgtttggcgtagtggctgccattacgccctggaatgtgcccatcatcctgctggtactgaaaatcgccccggccttgaaggctggcaataccgtggtcgccaagccatcggaatacaccccgctttctaccttgtacctgggtgaaattctgaaagatgtatttccgcccggcgtgctgaacgtgatagccggtgacggtcaggtgggggcgcgcctggcatcgcatccgctggtgcagaaggtgacgttcaccggcagcgtggcaaccggaaaaaaactctatgccagcgccgcgcaggatgtaaaacgcctgacgctggaactgggcggtaacgatgcggccatcgtgctggacgatgccaatgtcgatgccattgccgagaagattttctggggcgccttctggaatagcggtcaggtgtgctttgccatcaagcgcctctatgtgcacgagcgtgttttccagcccttgctcgatgccctggtgaaacgcgcgcaaaaaacccgcgtgggcgatggccagctgccgggtaccgagctggggccgcttaccaacaaagcccagtttgagcgcgtgatatcgctggtggaagacgccagacgccatggcgccaccattcattcaggcggtgctgcattgcctggccccggctatttctatccgcccaccctggtcaccggcataggcgcaggtgtcgcgctggtggatgaagagcagttcggaccagtattgccgctgattcctttccgtgatgagcaagaggcggtgcgtcaggccaacgacagtccgtttggtctgggcgcttcggtttggaccgccaatcccgaacgcggcctggcgctggtacgccagctccaggccgggctcgcctgggtcaaccagcatggcgatatccatcccggtgcgcccaagggcggctacaaatccagtggccttggctacgagggcgggctgcgtggctatgacgagttcagcgagctgcaagtcgtcaatgcggcgctggtttaa

SEQ ID NO: 4 - protein, 469 aa, Methylovorus glucosotrophus
MSTFHLLIDGHLQASDQSDVVINPATELEVGRAPRASATQVDQAVEAAHQAFHRWASQPEVRQQALLGAAAAIRQHADALARLITQEQGRPLHFTQGEVAGAAATFEHYAGFAAPSDVVLQQDEQKRVSIERRPFGVVAAITPWNVPIILLVLKIAPALKAGNTVVAKPSEYTPLSTLYLGEILKDVFPPGVLNVIAGDGQVGARLASHPLVQKVTFTGSVATGKKLYASAAQDVKRLTLELGGNDAAIVLDDANVDAIAEKIFWGAFWNSGQVCFAIKRLYVHERVFQPLLDALVKRAQKTRVGDGQLPGTELGPLTNKAQFERVISLVEDARRHGATIHSGGAALPGPGYFYPPTLVTGIGAGVALVDEEQFGPVLPLIPFRDEQEAVRQANDSPFGLGASVWTANPERGLALVRQLQAGLAWVNQHGDIHPGAPKGGYKSSGLGYEGGLRGYDEFSELQVVNAALV

SEQ ID NO: 5 - DNA, 1410 bp, Pseudomonas multiresinivorans
  source 1..1410: mol_type = genomic DNA
atgtcgcgctatgaactgctgatcgatggtcgcctccaggcggccgagcactacgaccgggttatagacccggccagcgaagaactcgtcggcgaagccgcccgcgccagcctggagcaggtcgacgcggcggtggacgccgcgcaccgcgccttcccaacctgggccaccgatctcgacggccgccgccagagcctggcccgagccgccgaacgagtacgcgagaacgcccaggcgctggccgagctgatcacccgcgaacagggtcgcccgctgcgctcgacactggaggaagtggcgggcgtcgccgccactttcgagcaccacgcacatctggagcttcccgccgatacccagttgcgcgacgacggcgaacgcctggtgcgcatcacccgcaaacccctgggggtggtcgccgcaatcaccccgtggaacgtcccgctgatcctgctggtgctgaagatcgcgcccgccctgcatgccggcaacaccgtggtggccaagccctcggaacacacgccgctgtccaccctgctgctggcgcgactgctgggcgatgtgttccctgctggcgtgttcaacgtgattgccggtgcaggcgaggtcggcgaacacctggtgcgccatccccgagtgcgccacgtgaccttcaccggcagcgtcgccaccggcaagcgcctgtatgccggcgcagcggacgacctcaagcgcctgaccctggaactgggcggcaacgatgccgcgctggtgctggaagatgccgacctcgaagccatcgtcgaaccgctgttctggggcgccttctggaacagcggccaggtgtgcttcgcgatcaagcgcctgtacgtgcatgaaagcctgttcgaaccgctgctggccaaactcgccgaacgcgccgagcgcacccgcctcggccatgggctcgacccgcagacggaactggggccgctgaccaacgcgcagcaactggaacgggtcatcaccctggtggaagacgccaaggctcacggagcgcgcatccacagcggtggcacgcggcccgacggccccggttacttctacccgccgaccctggtcagcggcgtggcggccggtgtcgcgctggtggatgaggaacagttcggcccggtgctgccggtgatcccgttccgcgacgaagaggacgccatcgcccaggccaacgccagcccctacggcctcggcgcctcggtgtggacccgcgacctggcgcgcggcgaagccatcgccgaacggttggaggcgggcctggcctgggtcaaccagcacggccacatccagcccggcgcgcccaagggcgggcacaagtggagcgggctcggctacgaaggcgggcaacgcggttacgaggccttcagcgagctgcaggtgctcaacatttcgcggcgctga

SEQ ID NO: 6 - protein, 469 aa, Pseudomonas multiresinivorans
MSRYELLIDGRLQAAEHYDRVIDPASEELVGEAARASLEQVDAAVDAAHRAFPTWATDLDGRRQSLARAAERVRENAQALAELITREQGRPLRSTLEEVAGVAATFEHHAHLELPADTQLRDDGERLVRITRKPLGVVAAITPWNVPLILLVLKIAPALHAGNTVVAKPSEHTPLSTLLLARLLGDVFPAGVFNVIAGAGEVGEHLVRHPRVRHVTFTGSVATGKRLYAGAADDLKRLTLELGGNDAALVLEDADLEAIVEPLFWGAFWNSGQVCFAIKRLYVHESLFEPLLAKLAERAERTRLGHGLDPQTELGPLTNAQQLERVITLVEDAKAHGARIHSGGTRPDGPGYFYPPTLVSGVAAGVALVDEEQFGPVLPVIPFRDEEDAIAQANASPYGLGASVWTRDLARGEAIAERLEAGLAWVNQHGHIQPGAPKGGHKWSGLGYEGGQRGYEAFSELQVLNISRR

SEQ ID NO: 7 - DNA, 1521 bp, Raoultella ornithinolytica
  source 1..1521: mol_type = genomic DNA
atgcgttatgcacatcctggcaccccgggcgccttagtttcattcaagtccgcatacggtaactatattgacggtcaatttgtcgaaccgctcggcggcgaatactttatgaatacctcccccgtggacgggagtgacattgcacaatttccccgctccgatgccaaagatatcgattttgctcttgatgccgcacaccgcgccgcggaagcctgggggaaaacatcggtacagcatcgttccaacctgctgcttcaggtcgccgatcggattcaggagaacctggaatatctggcgattgctgaaagctgggacaatggtaaaccggtgcgcgaaacgctgaatgccgatctgccgttggcggtcgatcacttccgctattttgccggctgtctgcgggcacaggaggggagtactgcggaaattgatgaaaccaccgtggcctatcacttccatgaaccgctgggcgtagtcgggcaaattattccgtggaactttccgctgctgatggcggcctggaagctggcgccggcgctggcggccgggaactgtgtggtgctcaagccggcagagcagacgccgctgagcatcacgctgctgctggaaattattggcgacctcttcccgccgggcgtcctgaacgtggtgcagggcttcggtaaagaggccggtgaagcgctggcaaccagcaagcgtattgccaaaattgcctttaccggctcaacgcccgtcggacggcatattctggcctgcgcggcggagaacattattcccgccaccgttgagctgggcggcaagtcgccaaatatctattttgccgatgtgatggacggagaagaagagtttatcgagaaggcggtggaggggctggtgctgggcttcttcaaccagggcgaagtatgtacctgcccatcgcgcgccctgatccatgaatccatctacgagccgtttatggagcgagtgatggcgaaggtggcccagattcgccgcggcgatccctttgataccgacaccatgatcggggcacaggcatcacgccagcagttcgataagatcctgtcgtacattaagattgcccgcgaagagggggggcagatcctgaccggcggagaacgcgccagtattacggctgaactggataatggttactacattcagccaactctgattaaggggcgcaatgatatgcgcagcttccaggaagagatttttggcccggtcatcggcgtcacgaccttcaaagatgaggcagaagcgctggaaatagccaaccagactcagtttgggctcggcgccggcgtctggacccgcgacagcaatctggcgtaccgaatggggcgtgggattaaagccggtcgtgtctggaccaactgttatcacgtctacccggcccatgccgcgtttggcggctataaacagtcaggcgtcggtcgtgaaactcataaaatggcccttgatgcctatcaacagacgaaaaacctgctggtgagctacggtaccgcgccgttaggactgttttaa

SEQ ID NO: 8 - protein, 506 aa, Raoultella ornithinolytica
MRYAHPGTPGALVSFKSAYGNYIDGQFVEPLGGEYFMNTSPVDGSDIAQFPRSDAKDIDFALDAAHRAAEAWGKTSVQHRSNLLLQVADRIQENLEYLAIAESWDNGKPVRETLNADLPLAVDHFRYFAGCLRAQEGSTAEIDETTVAYHFHEPLGVVGQIIPWNFPLLMAAWKLAPALAAGNCVVLKPAEQTPLSITLLLEIIGDLFPPGVLNVVQGFGKEAGEALATSKRIAKIAFTGSTPVGRHILACAAENIIPATVELGGKSPNIYFADVMDGEEEFIEKAVEGLVLGFFNQGEVCTCPSRALIHESIYEPFMERVMAKVAQIRRGDPFDTDTMIGAQASRQQFDKILSYIKIAREEGGQILTGGERASITAELDNGYYIQPTLIKGRNDMRSFQEEIFGPVIGVTTFKDEAEALEIANQTQFGLGAGVWTRDSNLAYRMGRGIKAGRVWTNCYHVYPAHAAFGGYKQSGVGRETHKMALDAYQQTKNLLVSYGTAPLGLF

SEQ ID NO: 9 - DNA, 1452 bp, Comamonas testosteroni
  source 1..1452: mol_type = genomic DNA
atgatcgaacaaaaaatgctgatcgccggccaggaatgtgcagccggcaatggcgcaacgtttgagcgcaagaatccgctggatggatccgtcgccacacgcgccccggcagccacgaccgaggatgcgattcgcgcctgcgacgctgctgcagccgccttccccgcctggtcgcaactggggccgaacgcccgccgcgccatgctgatgaaggcctcgcaggcactggaagccaagggcgaagcgattgctgcggccatggctgccgagaccggcgcctcgggcatctgggccggcttcaacgtgcatctggccgccagcatgctgctggaggcggcttcgctgaccacgcagatcaatggcgagatcattccctccgacgtacccggcagcgtggccatggccgtgcgccagcccgccggcgtggtactcggtatcgcgccctggaatgctcccgtgatcctggccgtgcgcagcatctccacggccctggcctgcggcaacaccgtgattctcaagggctcggaactctgccccgccacccacggcctgatcatcgaggcactgcaggacgcaggcctgcccgccggcgtggtgaactttgtgaccaatgcgcccgccgatgcgggcagcgtggtcgaagccatcgtggcccacccggccgtgcgccgcgtgagctttaccggctccaccaaggtgggccgcatcatcggccagacctgcgccaggcacttgaagcctgcgctgctggagcttggcggcaaggcccccttcctggtgctcgacgatgccgatatcgatgcggccgtgaacgccgccacctttggcgcgtttgccaactcgggccagatctgcatgtctaccgagcgctttgtggtggataacaaggtggccgacgagttcatcgccaagtttgccgccaaggccagcagcctgccgctgggcgacccgcgcaagggccccgtggtgctgggctcggtcgtcgatctggctacggtggagcgctgcaatgccatgatcgacgacgcgctggccaagggcgcaaaaatcgtctgcggcggcaaggccgagagcacgctgatgcccgccacgctgatcgaccatgtgacgccggcgatgcgcatattccacgaggagacctttggcccggtcaaaggcatcgtgcgcgtgaacggcgaggaagaagccattgccacggccaatgacaacgagttcggtctgtcctccgcagtcttcacccgggacacggcccgcggctggcgtgtggcggcacgcatcgaggccggcatctgccacatcaacggccccacggtgcatgacgaagcccagatgccgtttggtggcgtcaaggcctcgggctatggccatttcgggggccagcagggcatcaatgcctttaccgaaacccgctgggtgaccatgcagaccgcagaacgccactatccgttctaa

SEQ ID NO: 10 - protein, 483 aa, Comamonas testosteroni
MIEQKMLIAGQECAAGNGATFERKNPLDGSVATRAPAATTEDAIRACDAAAAAFPAWSQLGPNARRAMLMKASQALEAKGEAIAAAMAAETGASGIWAGFNVHLAASMLLEAASLTTQINGEIIPSDVPGSVAMAVRQPAGVVLGIAPWNAPVILAVRSISTALACGNTVILKGSELCPATHGLIIEALQDAGLPAGVVNFVTNAPADAGSVVEAIVAHPAVRRVSFTGSTKVGRIIGQTCARHLKPALLELGGKAPFLVLDDADIDAAVNAATFGAFANSGQICMSTERFVVDNKVADEFIAKFAAKASSLPLGDPRKGPVVLGSVVDLATVERCNAMIDDALAKGAKIVCGGKAESTLMPATLIDHVTPAMRIFHEETFGPVKGIVRVNGEEEAIATANDNEFGLSSAVFTRDTARGWRVAARIEAGICHINGPTVHDEAQMPFGGVKASGYGHFGGQQGINAFTETRWVTMQTAERHYPF

SEQ ID NO: 11 - DNA, 1521 bp, Corynebacterium glutamicum
  source 1..1521: mol_type = genomic DNA
atgactgtctacgcaaatccaggaaccgaaggctcgatcgttaactatgaaaagcgctacgagaactacattggtggcaagtgggttccaccggtagagggccagtaccttgagaacatttcacctgtcactggtgaagttttctgtgaggtcgcacgtggcaccgcagcggacgtggagcttgcactggatgctgcacatgcagccgctgatgcgtggggcaagacttctgtcgctgaacgtgctctgatcctgcaccgcattgcggaccgcatggaagagcacctggaagaaatcgcagttgcagaaacctgggagaacggcaaggcagtccgtgagactcttgctgcagatatcccactggcaatcgaccacttccgctactttgctggcgcgatccgtgctcaggaagatcgttcctcacagatcgaccacaacactgttgcttaccacttcaacgagccaatcggtgttgttggtcagatcattccttggaacttcccaatcctcatggctacctggaagctcgcaccggcacttgctgcaggtaacgcgatcgtcatgaagccagctgagcagaccccagcatccattttgtatctgattaacatcatcggcgatctcatcccagagggcgtcctcaacatcgtcaacggactcggcggtgaagcaggcgctgcactgtccggctctaatcggattggcaagattgctttcaccggttccaccgaggtcggcaagctgatcaaccgcgctgcatccgacaagatcattcctgtcaccctggagctcggcggtaagtccccatccatcttcttctccgatgttctgtcacaggatgacgccttcgcagagaaggcagttgaaggcttcgcgatgttcgccctcaatcagggtgaagtttgtacctgtccttcccgtgcacttgttcatgagtccatcgctgatgaattcctcgagcttggcgtgaagcgagttcagaacatcaagctgggtaacccacttgatactgaaaccatgatgggtgctcaggcgtcccaggagcagatggacaagatctcctcctacctgaagatcggcccagaagaaggcgctcaaaccctcactggtggcaaggtcaacaaggttgatggcatggagaacggttactacattgagccaaccgttttccgcggcaccaacgacatgaggatcttccgcgaggaaatcttcggaccagtcctttctgttgctaccttcagcgacttcgatgaggccatccgtattgcaaacgacaccaactacggcctcggcgctggtgtctggagccgtgaccaaaacaccatttatcgtgcaggtcgcgcaatccaggctggtcgagtttgggtcaaccagtaccacaactacccagcgcactccgctttcggtggatacaaggagtccggcatcggccgtgagaaccacctcatgatgctgaaccactaccagcagaccaagaacctgttggtctcctacgatccaaacccaaccggactgttctaa

SEQ ID NO: 12 - protein, 506 aa, Corynebacterium glutamicum
MTVYANPGTEGSIVNYEKRYENYIGGKWVPPVEGQYLENISPVTGEVFCEVARGTAADVELALDAAHAAADAWGKTSVAERALILHRIADRMEEHLEEIAVAETWENGKAVRETLAADIPLAIDHFRYFAGAIRAQEDRSSQIDHNTVAYHFNEPIGVVGQIIPWNFPILMATWKLAPALAAGNAIVMKPAEQTPASILYLINIIGDLIPEGVLNIVNGLGGEAGAALSGSNRIGKIAFTGSTEVGKLINRAASDKIIPVTLELGGKSPSIFFSDVLSQDDAFAEKAVEGFAMFALNQGEVCTCPSRALVHESIADEFLELGVKRVQNIKLGNPLDTETMMGAQASQEQMDKISSYLKIGPEEGAQTLTGGKVNKVDGMENGYYIEPTVFRGTNDMRIFREEIFGPVLSVATFSDFDEAIRIANDTNYGLGAGVWSRDQNTIYRAGRAIQAGRVWVNQYHNYPAHSAFGGYKESGIGRENHLMMLNHYQQTKNLLVSYDPNPTGLF

SEQ ID NO: 13 - DNA, 1014 bp, Geobacillus stearothermophilus
  source 1..1014: mol_type = genomic DNA
atgaaagctgcagttgtggaacaatttaaaaagccgttacaagtgaaagaagtggaaaaacctaagatctcatacggggaagtattagtgcgcatcaaagcgtgtggggtatgccatacagacttgcatgccgcacatggcgactggcctgtaaagcctaaactgcctctcattcctggccatgaaggcgtcggtgtaattgaagaagtaggtcctggggtaacacatttaaaagttggagatcgcgtaggtatcccttggctttattcggcgtgcggtcattgtgactattgcttaagcggacaagaaacattatgcgaacgtcaacaaaacgctggctattccgtcgatggtggttatgctgaatattgccgtgctgcagccgattatgtcgtaaaaattcctgataacttatcgtttgaagaagccgctccaatcttttgcgctggtgtaacaacatataaagcgctcaaagtaacaggcgcaaaaccaggtgaatgggtagccatttacggtatcggcgggcttggacatgtcgcagtccaatacgcaaaggcgatggggttaaacgtcgttgctgtcgatttaggtgatgaaaaacttgagcttgctaaacaacttggtgcagatcttgtcgtcaatccgaaacatgatgatgcagcacaatggataaaagaaaaagtgggcggtgtgcatgcgactgtcgtcacagctgtttcaaaagccgcgttcgaatcagcctacaaatccattcgtcgcggtggtgcttgcgtactcgtcggattaccgccggaagaaatacctattccaattttcgatacagtattaaatggagtaaaaattattggttctatcgttggtacgcgcaaagacttacaagaggcacttcaatttgcagcagaaggaaaagtaaaaacaattgtcgaagtgcaaccgcttgaaaacattaacgacgtattcgatcgtatgttaaaagggcaaattaacggccgcgtcgtgttaaaagtagattaa

SEQ ID NO: 14 - protein, 337 aa, Geobacillus stearothermophilus
MKAAVVEQFKKPLQVKEVEKPKISYGEVLVRIKACGVCHTDLHAAHGDWPVKPKLPLIPGHEGVGVIEEVGPGVTHLKVGDRVGIPWLYSACGHCDYCLSGQETLCERQQNAGYSVDGGYAEYCRAAADYVVKIPDNLSFEEAAPIFCAGVTTYKALKVTGAKPGEWVAIYGIGGLGHVAVQYAKAMGLNVVAVDLGDEKLELAKQLGADLVVNPKHDDAAQWIKEKVGGVHATVVTAVSKAAFESAYKSIRRGGACVLVGLPPEEIPIPIFDTVLNGVKIIGSIVGTRKDLQEALQFAAEGKVKTIVEVQPLENINDVFDRMLKGQINGRVVLKVD

SEQ ID NO: 15 - DNA, 1062 bp, Galactocandida mastotermitis
  source 1..1062: mol_type = genomic DNA
atgagcacaccggaaaatctgagctttgtgctgcagaaaccgtttgatgtgaaatttgaagatcgtccgattccgaaactgagcgatccgtatagcgttaaaattcaggtgaaaaaaaccggcatttgcggtagtgatgttcactatttcacccatggtgcaattggtgattttgttgttaaagcaccgatggttctgggtcatgaaagcagcggtgttgttctggaagttggtagcgaagttaaaagcctgaaagttggtgatcgtgttgcaatggaaccgggtgttccgagccgtcatagtgatgagtataaaagcggtcgttataatctgtgtccgcacatggcatttgcagcaacccctccgtatgatggcaccctgtgtaaatactatattctgccggaagatttctgcgttaaactgccggaacatgttagcctggaagaaggtgcactggttgaaccgctgagcgttgcagttcatagcagcaaactgggtaacattaaaccgggtagccatgttgcaatttatggtgcaggtccggttggtctgctggttgcagcagttgcaagcgcatttggtgcagaaagcgttaccattattgatctggttgaaagccgtctgaatctggcaaaagaactgggtgcaaccgcaaccgttcaggttgattttaaagataccccgaaagaaagcgcagcaaaagttgttgcagcaaataatggcattgcaccggatgttgttattgatgcaagcggtgcagaagcaagcattaattcagccattaatgcaattcgtccgggtggcacctatgttcaggtgggtatgggtaaaccggatgtgagctttccgattgcaaccctgattggtaaagaactgaccgttaaaggtagctttcgttatggttatggtgattatccgctggcagttagcctgctggcaagcggtaaagttaatgtgaaaaaactgatcacccatgaagtgaaattcgaggatgcagcagaagcatttcagctggttcgtgatggtaaagccattaaatgtattatcaacggtccggaataa

SEQ ID NO: 16 - protein, 353 aa, Galactocandida mastotermitis
MSTPENLSFVLQKPFDVKFEDRPIPKLSDPYSVKIQVKKTGICGSDVHYFTHGAIGDFVVKAPMVLGHESSGVVLEVGSEVKSLKVGDRVAMEPGVPSRHSDEYKSGRYNLCPHMAFAATPPYDGTLCKYYILPEDFCVKLPEHVSLEEGALVEPLSVAVHSSKLGNIKPGSHVAIYGAGPVGLLVAAVASAFGAESVTIIDLVESRLNLAKELGATATVQVDFKDTPKESAAKVVAANNGIAPDVVIDASGAEASINSAINAIRPGGTYVQVGMGKPDVSFPIATLIGKELTVKGSFRYGYGDYPLAVSLLASGKVNVKKLITHEVKFEDAAEAFQLVRDGKAIKCIINGPE